European Patent Specification EP 4 010 467 B1, published April 24, 2024. Title: Protein. Applicant: GlaxoSmithKline Biologicals S.A. The sequence listing filed with the application follows.

SEQUENCE LISTING (15 sequences)

SEQ ID NO: 1 - protein, 713 aa, Campylobacter jejuni
MLKKEYLKNPYLVLFAMIILAYVFSVFCRFYWVWWASEFNEYFFNNQLMIISNDGYAFAEGARDMIAGFHQPNDLSYYGSSLSALTYWLYKITPFSFESIILYMSTFLSSLVVIPTILLANEYKRPLMGFVAALLASIANSYYNRTMSGYYDTDMLVIVLPMFILFFMVRMILKKDFFSLIALPLFIGIYLWWYPSSYTLNVALIGLFLIYTLIFHRKEKIFYIAVILSSLTLSNIAWFYQSAIIVILFALFALEQKRLNFMIIGILGSATLIFLILSGGVDPILYQLKFYIFRSDESANLTQGFMYFNVNQTIQEVENVDLSEFMRRISGSEIVFLFSLFGFVWLLRKHKSMIMALPILVLGFLALKGGLRFTIYSVPVMALGFGFLLSEFKAIMVKKYSQLTSNVCIVFATILTLAPVFIHIYNYKAPTVFSQNEASLLNQLKNIANREDYVVTWWDYGYPVRYYSDVKTLVDGGKHLGKDNFFPSFALSKDEQAAANMARLSVEYTEKSFYAPQNDILKTDILQAMMKDYNQSNVDLFLASLSKPDFKIDTPKTRDIYLYMPARMSLIFSTVASFSFINLDTGVLDKPFTFSTAYPLDVKNGEIYLSNGVVLSDDFRSFKIGDNVVSVNSIVEINSIKQGEYKITPIDDKAQFYIFYLKDSAIPYAQFILMDKTMFNSAYVQMFFLGNYDKNLFDLVINSRDAKVFKLKI

SEQ ID NO: 2 - protein, 713 aa, Campylobacter jejuni
MLKKEYLKNPYLVLFAMIILAYVFSVFCRFYWVWWASEFNEYFFNNQLMIISNDGYAFAEGARDMIAGFHQPNDLSRYGSSLSALTYWLYKITPFSFESIILYMSTFLSSLVVIPTILLANEYKRPLMGFVAALLASIANSYYNRTMSGYYDTDMLVIVLPMFILFFMVRMILKKDFFSLIALPLFIGIYLWWYPSSYTLNVALIGLFLIYTLIFHRKEKIFYIAVILSSLTLSNIAWFYQSAIIVILFALFALEQKRLNFMIIGILGSATLIFLILSGGVDPILYQLKFYIFRSDESANLTQGFMYFNVVQTIQEVENVDLSEFMRRISGSEIVFLFSLFGFVWLLRKHKSMIMALPILVLGFLALKGGLRFTIYSVPVMALGFGFLLSEFKAIMVKKYSQLTSNVCIVFATILTLAPVFIHIYNYKAPTVFSQNEASLLNQLKNIANREDYVVTWWDYGYPVRYYSDVKTLVDGGKHLGKDNFFPSFALSKDEQAAANMARLSVEYTEKSFYAPQNDILKTDILQAMMKDYNQSNVDLFLASLSKPDFKIDTPKTRDIYLYMPARMSLIFSTVASFSFINLDTGVLDKPFTFSTAYPLDVKNGEIYLSNGVVLSDDFRSFKIGDNVVSVNSIVEINSIKQGEYKITPIDDKAQFYIFYLKDSAIPYAQFILMDKTMFNSAYVQMFFLGNYDKNLFDLVINSRDAKVFKLKI

SEQ ID NO: 3 - protein, 713 aa, Campylobacter jejuni
MLKKEYLKNPYLVLFAMIILAYVFSVFCRFYWVWWASEFNEYFFNNQLMIISNDGYRFAEGARDMIAGFHQPNDLSRYGSSLSALTYWLYKITPFSFESIILYMSTFLSSLVVIPTILLANEYKRPLMGFVAALLASIANSYYNRTMSGYYDTDMLVIVLPMFILFFMVRMILKKDFFSLIALPLFIGIYLWWYPSSYTLNVALIGLFLIYTLIFHRKEKIFYIAVILSSLTLSNIAWFYQSAIIVILFALFALEQKRLNFMIIGILGSATLIFLILSGGVDPILYQLKFYIFRSDESANLTQGFMYFNVVQTIQEVENVDLSEFMRRISGSEIVFLFSLFGFVWLLRKHKSMIMALPILVLGFLALKGGLRFTIYSVPVMALGFGFLLSEFKAIMVKKYSQLTSNVCIVFATILTLAPVFIHIYNYKAPTVFSQNEASLLNQLKNIANREDYVVTWWDYGYPVRYYSDVKTLVDGGKHLGKDNFFPSFALSKDEQAAANMARLSVEYTEKSFYAPQNDILKTDILQAMMKDYNQSNVDLFLASLSKPDFKIDTPKTRDIYLYMPARMSLIFSTVASFSFINLDTGVLDKPFTFSTAYPLDVKNGEIYLSNGVVLSDDFRSFKIGDNVVSVNSIVEINSIKQGEYKITPIDDKAQFYIFYLKDSAIPYAQFILMDKTMFNSAYVQMFFLGNYDKNLFDLVINSRDAKVFKLKI

SEQ ID NO: 4 - protein, 713 aa, Campylobacter jejuni
MLKKEYLKNPYLVLFAMIILAYVFSVFCRFYWVWWASEFNEYFFNNQLMIISNDGYRFAEGARDMIAGFHQPNDLSRYGSSLSALTYWLYKITPFSFESIILYMSTFLSSLVVIPTILLANEYKRPLMGFVAALLASIANSYYNRTMSGYYDTDMLVIVLPMFILFFMVRMILKKDFFSLIALPLFIGIYLWWYPSSYTLNVALIGLFLIYTLIFHRKEKIFYIAVILSSLTLSNIAWFYQSAIIVILFALFALEQKRLNFMIIGILGSATLIFLILSGGVDPILYQLKFYIFRSDESALPTQGFMYWNVVQTIQEVENVDLSEFMRRISGSEIVFLFSLFGFVWLLRKHKSMIMALPILVLGFLALKGGLRFTIYSVPVMALGFGFLLSEFKAIMVKKYSQLTSNVCIVFATILTLAPVFIHIYNYKAPTVFSQNEASLLNQLKNIANREDYVVTWWDYGWPVRYYSDVKTLVDGGKMLGKDNFFPSFALSKDEQAAANMARLSVEYTEKSFYAPQNDILKTDILQAMMKDYNQSNVDLFLASLSKPDFKIDTPKTRDIYLYMPARMSRIFSTVASFSFINLDTGVLDKPFTFSTAYPLDVKNGEIYLSNGVVLSDDFRSFKIGDNVVSVNSIVEINSIKQGEYKITPIDDKAQFYIFYLKDSAIPYAQFILMDKTMFNSAYVQMFFLGNYDKNLFDLVINSRDAKVFKLKI

SEQ ID NO: 5 - protein, 713 aa, Campylobacter jejuni
MLKKEYLKNPYLVLFAMIILAYVFSVFCRFYWVWWASEFNEYFFNNQLMIISNDGYRFAEGARDMIAGFHQPNDLSRYGSSLSALTYWLYKITPFSFESIILYMSTFLSSLVVIPTILLANEYKRPLMGFVAALLASIANSYYNRTMSGYYDTDMLVIVLPMFILFFMVRMILKKDFFSLIALPLFIGIYYWWYPSSYTLNVALIGLFLIYTLIFHRKEKIFYIAVILSSLTLSNIAWFYQSAIIVILFALFALEQKRLNFMIIGILGSATLIFLILSGGVDPILQQLKFYIFRLDESALPTQGFMYWNVVQTIQEVENVDLSEFMRRISGSEIVFLFSLFGFVWLLRKHKSMIMALPILVLGFLALKGGLRFTIYSVPVMSLGFGFLLSEFKAIMVKKYSQLTSNVCIVFATILTLAPVFIHIYNYKAPTVFSQNEASLLNQLKNIANREDYVVTWWDYGWPVRYYSDVKTLVDGGKMLGRDNFFPSFALSKDEQAAANMARLSVEYTEKSFYAPQNDILKRDILQAMMKDYNQSNVDLFLASLSKPDFKIDTPKTRDIYLYMPARMSRIFSTVASFSFINLDTGVLDKPFTFSTAYPLDVKNGEIYLSNGVVLSDDFRSFKIGDNVVSVNSIVEINSIKQGEYKITPIDDKAQFYIFYLKDSAIPYAQFILMDKTMFNSAYVQMFFLGNYDKNLFDLVINSRDAKVFKLKI

SEQ ID NO: 6 - protein, 713 aa, Campylobacter jejuni
MLKKEYLKNPYLVLFAMIILAYVFSVFCRFYWVWWASEFNEYFFNNQLMIISNDGYRFAEGARDMIAGFHQPNDLSRYGSSLSALTYWLYKITPFSFESIILYMSTFLSSLVVIPTILLANEYKRPLMGFVAALLASIANSYYNRTMSGYYDTDMLVIVLPMFILFFMVRMILKKDFFSLIALPLFIGIYYWWYPSSYTLNVALIGLFLIYTLIFHRKEKIFYIAVILSSLTLSNIAWFYQSAIIVILFALFALEQKRLNFMIIGILGSATLIFLILSGGVDPILQQLKFYIFRLDRSALPTQGFMYWNVVQTIQEVENVDLSEFMRRISGSEIVFLFSLFGFVWLLRKHKSMIMALPILVLGFLALKGGLRFTIYSVPVMSLGFGFLLSEFKAIMVKKYSQLTSNVCIVFATILTLAPVFIHIYNYKAPTVFSQNEASLLNQLKNIANREDYVVTWWDYGWPVRYYSDVKTLVDGGKMLGRDNFFPSFALSKDEQAAANMARLSVEYTEKSFYAPQNDILKRDILQAMMKDYNQSNVDLFLASLSKPDFKIDTPKTRDIYLYMPARMSRIFSTVASFSFINLDTGVLDKPFTFSTAYPLDVKNGEIYLSNGVVLSDDFRSFKIGDNVVSVNSIVEINSIKQGEYKITPIDDKAQFYIFYLKDSAIPYAQFILMDKTMFNSAYVQMFFLGNYDKNLFDLVINSRDAKVFKLKI

SEQ ID NO: 7 - protein, 713 aa, Campylobacter jejuni
MLKKEYLKNPYLVLFAMIILAYVFSVFCRFYWVWWASEFNEYFFNNQLMIISNDGYRFAEGARDMIAGFHQPNDLSRYGDSLSALTYWLYKITPFSFESIILYMSTFLSSLVVIPTILLANEYKRPLMGFVAALLASIANSYYNRTMSGYYDTDMLVIVLPMFILFFMVRMILKKDFFSLIALPLFIGIYYWWYPSSYTLNVALIGLFLIYTLIFHRKEKIFYIAVILSSLTLSNIAWFYQSAIIVILFALFALEQKRLNFMIIGILGSATLIFLILSGGVDPILQQLKFYIFRLDRSALPTQGFMYWNVVQTIQEVENVDLSEFMRRISGSEIVFLFSLFGFVWLLRKHKSMIMALPILVLGFLALKGGLRFTIYSVPVMSLGFGFLLSEFKAIMVKKYSQLTSNVCIVFATILTLAPVFIHIYNYKAPTVFSQNEASLLNQLKNIANREDYVVTWWDYGWPVRYYSDVKTLVDGGKMLGRDNFFPSFALSKDEQAAANMARLSVEYTEKSFYAPQNDILKRDILQAMMKDYNQSNVDLFLASLSKPDFKIDTPKTRDIYLYMPARMSRIFSTVASFSFINLDTGVLDKPFTFSTAYPLDVKNGEIYLSNGVVLSDDFRSFKIGDNVVSVNSIVEINSIKQGEYKITPIDDKAQFYIFYLKDSAIPYAQFILMDKTMFNSAYVQMFFLGNYDKNLFDLVINSRDAKVFKLKI

SEQ ID NO: 8 - protein, 713 aa, Campylobacter jejuni
MLKKEYLKNPYLVLFAMIILAYVFSVFCRFYWVWWASEFNEYFFNNQLMIISNDGYRFAEGARDMIAGFHQPNDLSRYGDSLSALTYWLYKITPFSFESIILYMSTFLSSLVVIPTILLANEYKRPLMGFVAALLASIANSYYNRTMSGYYDTDMLVIVLPMFILFFMVRMILKKDFFSLIALPLFVGIYYWWYPSSYTLNVALIGLFLIYTLIFHRKEKIFYIAVILSSLTLSNIAWFYQSAIIVILFALFALEQKRLNFMIIGILGSATLIFLILSGGVDPILQQLKFYIFRLDRSALPTQGFMYWNVVQTIQEVENVDLSEFMRRISGSEIVFLFSLFGFVWLLRKHKSMIMALPQLVLGFLALKGGLRFTIYSVPVMSLGFGFLLSEFKAIMVKKYSQLTSIVCIVFATILTLAPVFIHIYNYKAPTVFSQNEASLLNQLKNIANREDYVVTWWDYGWPVRYYSDVKTLVDGGKMLGRDNFFPSFALSKDEQAAANMARLSVEYTEKSFYAPQNDILKRDILQAMMKDYNQSNVDLFLASLSKPDFKIDTPKTRDIYLYMPARMSRIFSTVASFSFINLDTGVLDKPFTFSTAYPLDVKNGEIYLSNGVVLSDDFRSFKIGDNVVSVNSIVEINSIKQGEYKITPIDDKAQFYIFYLKDSAIPYAQFILMDKTMFNSAYVQMFFLGNYDKNLFDLVINSRDAKVFKLKI

SEQ ID NO: 9 - protein, 722 aa, Campylobacter jejuni
MLKKEYLKNPYLVLFAMIILAYVFSVFCRFYWVWWASEFNEYFFNNQLMIISNDGYAFAEGARDMIAGFHQPNDLSYYGSSLSALTYWLYKITPFSFESIILYMSTFLSSLVVIPTILLANEYKRPLMGFVAALLASIANSYYNRTMSGYYDTDMLVIVLPMFILFFMVRMILKKDFFSLIALPLFIGIYLWWYPSSYTLNVALIGLFLIYTLIFHRKEKIFYIAVILSSLTLSNIAWFYQSAIIVILFALFALEQKRLNFMIIGILGSATLIFLILSGGVDPILYQLKFYIFRSDESANLTQGFMYFNVNQTIQEVENVDLSEFMRRISGSEIVFLFSLFGFVWLLRKHKSMIMALPILVLGFLALKGGLRFTIYSVPVMALGFGFLLSEFKAIMVKKYSQLTSNVCIVFATILTLAPVFIHIYNYKAPTVFSQNEASLLNQLKNIANREDYVVTWWDYGYPVRYYSDVKTLVDGGKHLGKDNFFPSFALSKDEQAAANMARLSVEYTEKSFYAPQNDILKTDILQAMMKDYNQSNVDLFLASLSKPDFKIDTPKTRDIYLYMPARMSLIFSTVASFSFINLDTGVLDKPFTFSTAYPLDVKNGEIYLSNGVVLSDDFRSFKIGDNVVSVNSIVEINSIKQGEYKITPIDDKAQFYIFYLKDSAIPYAQFILMDKTMFNSAYVQMFFLGNYDKNLFDLVINSRDAKVFKLKIYPYDVPDYA

SEQ ID NO: 10 - protein, 712 aa, Campylobacter lari
MKLQQNFTDNNSIKYTCILILIAFAFSVLCRLYWVAWASEFYEFFFNDQLMITTNDGYAFAEGARDMIAGFHQPNDLSYFGSSLSTLTYWLYSILPFSFESIILYMSAFFASLIVVPIILIAREYKLTTYGFIAALLGSIANSYYNRTMSGYYDTDMLVLVLPMLILLTFIRLTINKDIFTLLLSPVFIMIYLWWYPSSYSLNFAMIGLFGLYTLVFHRKEKIFYLTIALMIIALSMLAWQYKLALIVLLFAIFAFKEEKINFYMIWALIFISILILHLSGGLDPVLYQLKFYVFKASDVQNLKDAAFMYFNVNETIMEVNTIDPEVFMQRISSSVLVFILSFIGFILLCKDHKSMLLALPMLALGFMALRAGLRFTIYAVPVMALGFGYFLYAFFNFLEKKQIKLSLRNKNILLILIAFFSISPALMHIYYYKSSTVFTSYEASILNDLKNKAQREDYVVAWWDYGYPIRYYSDVKTLIDGGKHLGKDNFFSSFVLSKEQIPAANMARLSVEYTEKSFKENYPDVLKAMVKDYNKTSAKDFLESLNDKDFKFDTNKTRDVYIYMPYRMLRIMPVVAQFANTNPDNGEQEKSLFFSQANAIAQDKTTGSVMLDNGVEIINDFRALKVEGASIPLKAFVDIESITNGKFYYNEIDSKAQIYLLFLREYKSFVILDESLYNSSYIQMFLLNQYDQDLFEQITNDTRAKIYRLKR

SEQ ID NO: 11 - protein, 713 aa, Campylobacter jejuni
MLKKEYLKNPYLVLFAMIILAYVFSVFCRFYWVWWASEFNEYFFNNQLMIISNDGYAFAEGARDMIAGFHQPNDLSHYGSSLSALTYWLYKITPFSFESIILYMSTFLSSLVVIPTILLANEYKRPLMGFVAALLASIANSYYNRTMSGYYDTDMLVIVLPMFILFFMVRMILKKDFFSLIALPLFIGIYLWWYPSSYTLNVALIGLFLIYTLIFHRKEKIFYIAVILSSLTLSNIAWFYQSAIIVILFALFALEQKRLNFMIIGILGSATLIFLILSGGVDPILYQLKFYIFRSDESANLTQGFMYFNVVQTIQEVENVDLSEFMRRISGSEIVFLFSLFGFVWLLRKHKSMIMALPILVLGFLALKGGLRFTIYSVPVMALGFGFLLSEFKAIMVKKYSQLTSNVCIVFATILTLAPVFIHIYNYKAPTVFSQNEASLLNQLKNIANREDYVVTWWDYGYPVRYYSDVKTLVDGGKHLGKDNFFPSFALSKDEQAAANMARLSVEYTEKSFYAPQNDILKTDILQAMMKDYNQSNVDLFLASLSKPDFKIDTPKTRDIYLYMPARMSLIFSTVASFSFINLDTGVLDKPFTFSTAYPLDVKNGEIYLSNGVVLSDDFRSFKIGDNVVSVNSIVEINSIKQGEYKITPIDDKAQFYIFYLKDSAIPYAQFILMDKTMFNSAYVQMFFLGNYDKNLFDLVINSRDAKVFKLKI

SEQ ID NO: 12 - protein, 714 aa, Campylobacter coli
MLKKEYFKNPTFILLAFIILAYVFSVLCRFYWIFWASEFNEYFFNNELMIISNDGYAFAEGARDMIAGFHQPNDLSYYGSSLSTLTYWFYKITPFSLESIFIYISTFLSSLVVIPLILIANEYKRPLMGFVAALLASIANSYYNRTMSGYYDTDMLVIVLAMMIVFFMIRLILKKDLLSLITLPLFVGIYLWWYPSSYTLNVALLGLFFIYTLVFHIKEKTLYMAIILASITLSNIAWFYQSAIIVILFSLFVLQNKRFSFALLGILGLATLVFLILSGGIDPILYQLKFYIFRSDESANLAQGFMYFNVNQTIQEVESIDLSIFMQRISGSELVFFVSLIGFIFLVRKHKSMILALPMLALGFLALKSGLRFTIYAVPVLALGFGFLMSLLQERKQKNNNTYWWANIGVFIFTFLSLIPMFYHINNYKAPTVFSQNEATKLDELKKIAQREDYVVTWWDYGYPIRYYSDVKTLADGGKHLGKDNFFPSFVLSKDQVAAANMARLSVEYTEKSFYAPLNDILKNDLLQAMMKDYNQNNVDLFLASLSKPDFKINMPKTRDVYIYMPARMSLIFSTVASFSFVDLETGEINKPFTFSAAYPLDVKNGEIYLSNGIALSDDFRSFKINNSTISVNSIIEINSIKQGEYKITPIDDMAQFYIFYLKDSTIPYAQFILMDKTMFNSAYVQMFFLGNYDKNLYDLVINARDAKVFKLKI

SEQ ID NO: 13 - protein, 711 aa, Campylobacter coli
MLKKEYFKNPTFILLTLIILAYAFSVLCRFYWVFWASEFNEYFFNNELMIISNDGYAFAEGARDMIAGFHQPNDLSYYGSSLSTLTYWFYKITPFSLESIFIYISTFLSSLVVVPLILIANEYKRPLMGFVAALLASIANSYYNRTMSGYYDTDMLVIVLAMMIVFFMIRLILRKDLLSLIALPLFVGIYLWWYPSSYTLNVALLGLLFIYTLVFHIKEKTLYMAIILASITLSNIAWFYQSAIIVILFSLFVLQNKRFSFALLGFLGLATLVFLILSGGVDPILYQLKFYIFRSDESANLAQGFMYFNVNQTIQEVESIDLSIFMKRISGSELVFFISLIGFIFLVRKHKSMILALPMLALGFLALKGGLRFTIYAVPVLALGFGFLMSLLQERKWKNKNIYWASVSIFTFLSLLPMFYHIINYKAPTVFSQNEASKLDELKKIAQREDYVVAWWDYGYPIRYYSDVKTLADGGKHLGKDNFFPSFILSKDQTAAANMARLSVEYTEKSFYAPSNDILKNDLLKAMMKDYKQNNVDLFLASLSKPDFKINTPKTRDVYIYMPARMSLIFSTVASFSFVDLDTGKIDKPFTFSAAYPLDVKNGEIYLSNGIVLSDDFRSFKINHNTIPVNSIIEVSSIKQGEYKITPIDDTAQFYILYLKDSTIPYAQFILMDKAMFNSAYVQMFFLGNYDKNLYDLVINTRDTKVFKLKI

SEQ ID NO: 14 - protein, 714 aa, Campylobacter coli
MLKKEYFKNPTFILLAFIILAYVFSVLCRFYWVFWASEFNEYFFNNELMIISNDGYAFAEGARDMIAGFHQPNDLSYYGSSLSTLTYWFYKITPFSLESIFIYISTFLSSLVVIPLILIANEYKRPLMGFVAALLASIANSYYNRTMSGYYDTDMLVIVLAMMIVFFMIRLILKKDLLSLIALPLFVGIYLWWYPSSYTLNVALLGLFFIYTLVFHIKEKTLYMAIILASITLSNIAWFYQSAIIVILFSLFVLQNKRFSFALLGILGLATLVFLILSGGIDPILYQLKFYIFRSDESANLAQGFMYFNVNQTIQEVESIDLSIFMQRISGSELVFFVSLIGFIFLVRKHKSMILALPMLALGFLALKSGLRFTIYAVPVLALGFGFLMSLLQERKQKNNNTYWWANIGVFIFTFLSLIPMFYHINNYKAPTVFSQNEATKLDELKKIAQREDYVVAWWDYGYPIRYYSDVKTLADGGKHLGKDNFFPSFVLSKDQVAAANMARLSVEYTEKSFYAPLNDILKNDLLQAMMKDYNQNNVDLFLALLSKPDFKINTPKTRDVYIYMPARMSLIFSTVASFSFVDLGTGEINKPFTFSAAYPLDVKNGEIYLSNGIVLSDDFRSFKINNSTISVNSIIEINSIKQGEYKITPIDDTAQFYIFYLKDSTIPYAQFILMDKTMFNSAYVQMFFLGNYDKNLYDLVINARDAKVFKLKF

SEQ ID NO: 15 - protein, 5 aa, Artificial
  Consensus sequence
  MISC_FEATURE (1)..(1): Xaa can be Asp or Glu
  MISC_FEATURE (2)..(2): Xaa can be any naturally occuring amino acid except proline
  MISC_FEATURE (4)..(4): Xaa can be any naturally occuring amino acid except proline
  MISC_FEATURE (5)..(5): Xaa can be Ser or Thr
XXNXX